European Patent Specification EP 3 565 823 B1, published May 29, 2024. Title: COMPOSITION. Applicant: Apitope International NV. The sequence listing filed with the application follows.

SEQUENCE LISTING (47 sequences)

SEQ ID NO: 1 - protein, 15 aa, Artificial Sequence
  Synthetic peptide
IFKKISRDKSVTIYL

SEQ ID NO: 2 - protein, 15 aa, Artificial Sequence
  Synthetic peptide
KGKKVYVTLTCAFRY

SEQ ID NO: 3 - protein, 22 aa, Artificial Sequence
  Synthetic peptide
VIGLTFRRDLYFSRVQVYPPVG

SEQ ID NO: 4 - protein, 37 aa, Artificial Sequence
  Synthetic peptide
ESLLKKLGSNTYPFLLTFPDYLPCSVMLQPAPQDSGK

SEQ ID NO: 5 - protein, 17 aa, Artificial Sequence
  Synthetic peptide
SSVRLLIRKVQHAPLEM

SEQ ID NO: 6 - protein, 26 aa, Artificial Sequence
  Synthetic peptide
AEAAWQFFMSDKPLHLAVSLNKEIYF

SEQ ID NO: 7 - protein, 41 aa, Artificial Sequence
  Synthetic peptide
LTKTLTLLPLLANNRERRGIALDGKIKHEDTNLASSTIIKE

SEQ ID NO: 8 - protein, 21 aa, Artificial Sequence
  Synthetic peptide
IDRTVLGILVSYQIKVKLTVS

SEQ ID NO: 9 - protein, 29 aa, Artificial Sequence
  Synthetic peptide
NTEKTVKKIKAFVEQVANVVLYSSDYYVK

SEQ ID NO: 10 - protein, 42 aa, Artificial Sequence
  Synthetic peptide
MAASGKTSKSEPNHVIFKKISRDKSVTIYLGNRDYIDHVSQV

SEQ ID NO: 11 - protein, 19 aa, Artificial Sequence
  Synthetic peptide
HVIFKKISRDKSVTIYLGN

SEQ ID NO: 12 - protein, 11 aa, Artificial Sequence
  Synthetic peptide
KKISRDKSVTI

SEQ ID NO: 13 - protein, 13 aa, Artificial Sequence
  Synthetic peptide
FKKISRDKSVTIY

SEQ ID NO: 14 - protein, 17 aa, Artificial Sequence
  Synthetic peptide
VIFKKISRDKSVTIYLG

SEQ ID NO: 15 - protein, 23 aa, Artificial Sequence
  Synthetic peptide
KKKVIFKKISRDKSVTIYLGKKK

SEQ ID NO: 16 - protein, 38 aa, Artificial Sequence
  Synthetic peptide
LTLLPLLANNRERRGIALDGKIKHEDTNLASSTIIKEG

SEQ ID NO: 17 - protein, 17 aa, Artificial Sequence
  Synthetic peptide
NRERRGIALDGKIKHED

SEQ ID NO: 18 - protein, 13 aa, Artificial Sequence
  Synthetic peptide
ERRGIALDGKIKH

SEQ ID NO: 19 - protein, 15 aa, Artificial Sequence
  Synthetic peptide
RERRGIALDGKIKHE

SEQ ID NO: 20 - protein, 20 aa, Artificial Sequence
  Synthetic peptide
DGKIKHEDTNLASSTIIKEG

SEQ ID NO: 21 - protein, 10 aa, Artificial Sequence
  Synthetic peptide
HEDTNLASST

SEQ ID NO: 22 - protein, 12 aa, Artificial Sequence
  Synthetic peptide
KHEDTNLASSTI

SEQ ID NO: 23 - protein, 14 aa, Artificial Sequence
  Synthetic peptide
IKHEDTNLASSTII

SEQ ID NO: 24 - protein, 16 aa, Artificial Sequence
  Synthetic peptide
KIKHEDTNLASSTIIK

SEQ ID NO: 25 - protein, 18 aa, Artificial Sequence
  Synthetic peptide
LTKTLTLLPLLANNRERR

SEQ ID NO: 26 - protein, 20 aa, Artificial Sequence
  Synthetic peptide
LTLLPLLANNRERRGIALDG

SEQ ID NO: 27 - protein, 10 aa, Artificial Sequence
  Synthetic peptide
LLANNRERRG

SEQ ID NO: 28 - protein, 12 aa, Artificial Sequence
  Synthetic peptide
PLLANNRERRGI

SEQ ID NO: 29 - protein, 14 aa, Artificial Sequence
  Synthetic peptide
LPLLANNRERRGIA

SEQ ID NO: 30 - protein, 15 aa, Artificial Sequence
  Synthetic peptide
NNRERRGIALDGKIK

SEQ ID NO: 31 - protein, 21 aa, Artificial Sequence
  Synthetic peptide
VKKIKAFVEQVANVVLYSSDY

SEQ ID NO: 32 - protein, 27 aa, Artificial Sequence
  Synthetic peptide
KKKVKKIKAFVEQVANVVLYSSDYKKK

SEQ ID NO: 33 - protein, 11 aa, Artificial Sequence
  Synthetic peptide
AFVEQVANVVL

SEQ ID NO: 34 - protein, 17 aa, Artificial Sequence
  Synthetic peptide
KKKAFVEQVANVVLKKK

SEQ ID NO: 35 - protein, 22 aa, Artificial Sequence
  Synthetic peptide
VIGLTFRRDLYFSRVQVYPPVG

SEQ ID NO: 36 - protein, 28 aa, Artificial Sequence
  Synthetic peptide
KKKVIGLTFRRDLYFSRVQVYPPVGKKK

SEQ ID NO: 37 - protein, 15 aa, Artificial Sequence
  Synthetic peptide
LTFRRDLYFSRVQVY

SEQ ID NO: 38 - protein, 21 aa, Artificial Sequence
  Synthetic peptide
KKKLTFRRDLYFSRVQVYKKK

SEQ ID NO: 39 - protein, 12 aa, Artificial Sequence
  Synthetic peptide
TFRRDLYFSRVQ

SEQ ID NO: 40 - protein, 10 aa, Artificial Sequence
  Synthetic peptide
RRDLYFSRVQ

SEQ ID NO: 41 - protein, 25 aa, Artificial Sequence
  Synthetic peptide
IDRTVLGILVSYQIKVKLTVSGFLG

SEQ ID NO: 42 - protein, 31 aa, Artificial Sequence
  Synthetic peptide
KKKIDRTVLGILVSYQIKVKLTVSGFLGKKK

SEQ ID NO: 43 - protein, 15 aa, Artificial Sequence
  Synthetic peptide
VLGILVSYQIKVKLT

SEQ ID NO: 44 - protein, 21 aa, Artificial Sequence
  Synthetic peptide
KKKVLGILVSYQIKVKLTKKK

SEQ ID NO: 45 - protein, 11 aa, Artificial Sequence
  Synthetic peptide
GILVSYQIKVK

SEQ ID NO: 46 - protein, 17 aa, Artificial Sequence
  Synthetic peptide
KKKGILVSYQIKVKKKK

SEQ ID NO: 47 - protein, 405 aa, Homo sapiens
MAASGKTSKSEPNHVIFKKISRDKSVTIYLGNRDYIDHVSQVQPVDGVVLVDPDLVKGKKVYVTLTCAFRYGQEDIDVIGLTFRRDLYFSRVQVYPPVGAASTPTKLQESLLKKLGSNTYPFLLTFPDYLPCSVMLQPAPQDSGKSCGVDFEVKAFATDSTDAEEDKIPKKSSVRLLIRKVQHAPLEMGPQPRAEAAWQFFMSDKPLHLAVSLNKEIYFHGEPIPVTVTVTNNTEKTVKKIKAFVEQVANVVLYSSDYYVKPVAMEEAQEKVPPNSTLTKTLTLLPLLANNRERRGIALDGKIKHEDTNLASSTIIKEGIDRTVLGILVSYQIKVKLTVSGFLGELTSSEVATEVPFRLMHPQPEDPAKESYQDANLVFEEFARHNLKDAGEAEEGKRDKNDVDE